European Patent Application EP 4 635 569 A2, published October 22, 2025. Title: METHODS OF DELIVERING A NEUROPROTECTIVE POLYPEPTIDE TO THE CENTRAL NERVOUS SYSTEM AND METHODS OF TREATING A CENTRAL NERVOUS SYSTEM DISEASE. Applicant: Peptron, Inc. Application EP, filed October 20, 2017. The sequence listing filed with the application follows.

SEQUENCE LISTING (55 sequences)

SEQ ID NO: 1 - protein, 30 aa, synthetic construct
  REGION 1..30: note = Description of Artificial Sequence: Note = Synthetic Construct
HAEGTFTSDVSSYLEGQAAKEFIAWLVKGR

SEQ ID NO: 2 - protein, 39 aa, synthetic construct
  REGION 1..39: note = Description of Artificial Sequence: Note = Synthetic Construct
HGEGTFTSDLSKQMEEEAVRLFIEWLKNGGPSSGAPPPS

SEQ ID NO: 3 - protein, 30 aa, synthetic construct
  REGION 1..30: note = Description of Artificial Sequence: Note = Synthetic Construct
HGEGTFTSDVSSYLEGQAAKEFIAWLVKGR

SEQ ID NO: 4 - protein, 30 aa, synthetic construct; identical to SEQ ID NO: 1
  REGION 1..30: note = Description of Artificial Sequence: Note = Synthetic Construct

SEQ ID NO: 5 - protein, 30 aa, synthetic construct
  REGION 1..30: note = Description of Artificial Sequence: Note = Synthetic Construct
HGEGTFTSDLSSYLEGQAAKEFIAWLVKGR

SEQ ID NO: 6 - protein, 30 aa, synthetic construct
  REGION 1..30: note = Description of Artificial Sequence: Note = Synthetic Construct
HGEGTFTSDLSKQMEGQAAKEFIAWLVKGR

SEQ ID NO: 7 - protein, 30 aa, synthetic construct
  REGION 1..30: note = Description of Artificial Sequence: Note = Synthetic Construct
HGEGTFTSDLSKQMEEEAVRLFIEWLKNGG

SEQ ID NO: 8 - protein, 31 aa, synthetic construct
  REGION 1..31: note = Description of Artificial Sequence: Note = Synthetic Construct
  VARIANT 2: note = Xaa= aminohexanoic acid
HXAEGTFTSDVSSYLEGQAAKEFIAWLVKGR

SEQ ID NO: 9 - protein, 39 aa, synthetic construct
  REGION 1..39: note = Description of Artificial Sequence: Note = Synthetic Construct
  VARIANT 30: note = Xaa=any amino acid
HAEGTFTSDVSSYLEGQAAKEFIAWLVKGXPSSGAPPPS

SEQ ID NO: 10 - protein, 39 aa, synthetic construct
  REGION 1..39: note = Description of Artificial Sequence: Note = Synthetic Construct
HAEGTFTSDLSKQMEEEAVRLFIEWLKNGGPSSGAPPPS

SEQ ID NO: 11 - protein, 30 aa, synthetic construct
  REGION 1..30: note = Description of Artificial Sequence: Note = Synthetic Construct
HAEGTFTSDLSKQMEEEAVRLFIEWLKNGG

SEQ ID NO: 12 - protein, 37 aa, synthetic construct
  REGION 1..37: note = Description of Artificial Sequence: Note = Synthetic Construct
HGEGTFTSDLSKQMEEEAVRLFIEWLKNGGPSSGAPP

SEQ ID NO: 13 - protein, 35 aa, synthetic construct
  REGION 1..35: note = Description of Artificial Sequence: Note = Synthetic Construct
HGEGTFTSDLSKQMEEEAVRLFIEWLKNGGPSSGA

SEQ ID NO: 14 - protein, 33 aa, synthetic construct
  REGION 1..33: note = Description of Artificial Sequence: Note = Synthetic Construct
HGEGTFTSDLSKQMEEEAVRLFIEWLKNGGPSS

SEQ ID NO: 15 - protein, 28 aa, synthetic construct
  REGION 1..28: note = Description of Artificial Sequence: Note = Synthetic Construct
HGEGTFTSDLSKQMEEEAVRLFIEWLKN

SEQ ID NO: 16 - protein, 26 aa, synthetic construct
  REGION 1..26: note = Description of Artificial Sequence: Note = Synthetic Construct
HGEGTFTSDLSKQMEEEAVRLFIEWL

SEQ ID NO: 17 - protein, 23 aa, synthetic construct
  REGION 1..23: note = Description of Artificial Sequence: Note = Synthetic Construct
HGEGTFTSDLSKQMEEEAVRLFI

SEQ ID NO: 18 - protein, 20 aa, synthetic construct
  REGION 1..20: note = Description of Artificial Sequence: Note = Synthetic Construct
HGEGTFTSDLSKQMEEEAVR

SEQ ID NO: 19 - protein, 17 aa, synthetic construct
  REGION 1..17: note = Description of Artificial Sequence: Note = Synthetic Construct
HGEGTFTSDLSKQMEEE

SEQ ID NO: 20 - protein, 14 aa, synthetic construct
  REGION 1..14: note = Description of Artificial Sequence: Note = Synthetic Construct
HGEGTFTSDLSKQM

SEQ ID NO: 21 - protein, 11 aa, synthetic construct
  REGION 1..11: note = Description of Artificial Sequence: Note = Synthetic Construct
HGEGTFTSDLS

SEQ ID NO: 22 - protein, 34 aa, synthetic construct
  REGION 1..34: note = Description of Artificial Sequence: Note = Synthetic Construct
  VARIANT 3..6: note = Xaa= aminohexanoic acid
HAXXXXEGTFTSDVSSYLEGQAAKEFIAWLVKGR

SEQ ID NO: 23 - protein, 38 aa, synthetic construct
  REGION 1..38: note = Description of Artificial Sequence: Note = Synthetic Construct
  VARIANT 3..10: note = Xaa=aminohexanoic acid
HAXXXXXXXXEGTFTSDVSSYLEGQAAKEFIAWLVKGR

SEQ ID NO: 24 - protein, 30 aa, synthetic construct
  REGION 1..30: note = Description of Artificial Sequence: Note = Synthetic Construct
HGEGTFTSDVSSYMEEQAVRLFIAWLVKGR

SEQ ID NO: 25 - protein, 30 aa, synthetic construct
  REGION 1..30: note = Description of Artificial Sequence: Note = Synthetic Construct
HGEGTFTSDVSSYMEEQAAKEFIAWLVKGR

SEQ ID NO: 26 - protein, 30 aa, synthetic construct
  REGION 1..30: note = Description of Artificial Sequence: Note = Synthetic Construct
HGEGTFTSDVSSYLEGQAVRLFIAWLVKGR

SEQ ID NO: 27 - protein, 30 aa, synthetic construct
  REGION 1..30: note = Description of Artificial Sequence: Note = Synthetic Construct
HGEGTFTSDVSKYLEGQAAKEFIAWLVKGR

SEQ ID NO: 28 - protein, 30 aa, synthetic construct
  REGION 1..30: note = Description of Artificial Sequence: Note = Synthetic Construct
HGEGTFTSDVSKYLEEEAAKEFIAWLVKGR

SEQ ID NO: 29 - protein, 30 aa, synthetic construct
  REGION 1..30: note = Description of Artificial Sequence: Note = Synthetic Construct
HGEGTFTSDVSKYLEEEAAKEFIEWLVKGG

SEQ ID NO: 30 - protein, 30 aa, synthetic construct
  REGION 1..30: note = Description of Artificial Sequence: Note = Synthetic Construct
HGEGTFTSDVSKYLEEEAAKEFIEWLVKGR

SEQ ID NO: 31 - protein, 30 aa, synthetic construct
  REGION 1..30: note = Description of Artificial Sequence: Note = Synthetic Construct
HGEGTFTSDLSKQMEEEAVRLFIEWLKNGR

SEQ ID NO: 32 - protein, 30 aa, synthetic construct
  REGION 1..30: note = Description of Artificial Sequence: Note = Synthetic Construct
HGEGTFTSDLSKQMEEEAVRLFIAWLKNGR

SEQ ID NO: 33 - protein, 30 aa, synthetic construct
  REGION 1..30: note = Description of Artificial Sequence: Note = Synthetic Construct
HGEGTFTSDLSKQMEEEAVREFIAWLKNGR

SEQ ID NO: 34 - protein, 39 aa, synthetic construct
  REGION 1..39: note = Description of Artificial Sequence: Note = Synthetic Construct
HGEGTFTSDVSSYLEGQAAKEFIAWLVKGGPSSGAPPPS

SEQ ID NO: 35 - protein, 39 aa, synthetic construct
  REGION 1..39: note = Description of Artificial Sequence: Note = Synthetic Construct
HGEGTFTSDVSSYLEGQAAKEFIEWLKNGGPSSGAPPPS

SEQ ID NO: 36 - protein, 30 aa, synthetic construct
  REGION 1..30: note = Description of Artificial Sequence: Note = Synthetic Construct
HGEGTFTSDVSSYLEEEAVRLFIAWLVKGR

SEQ ID NO: 37 - protein, 30 aa, synthetic construct
  REGION 1..30: note = Description of Artificial Sequence: Note = Synthetic Construct
HGEGTFTSDLSKQMEGQAAKEFIEWLKNGR

SEQ ID NO: 38 - protein, 42 aa, synthetic construct
  REGION 1..42: note = Description of Artificial Sequence: Note = Synthetic Construct
YGEGTFISDYSIAMDKIHQQDFVNWLLAQKGKKNDWKHNITQ

SEQ ID NO: 39 - protein, 39 aa, synthetic construct
  REGION 1..39: note = Description of Artificial Sequence: Note = Synthetic Construct
HGEGTFTSDVSSYLEGQAAKEFIAWLVKGRPSSGAPPPS

SEQ ID NO: 40 - protein, 42 aa, synthetic construct
  REGION 1..42: note = Description of Artificial Sequence: Note = Synthetic Construct
HGEGTFTSDVSSYLEGQAAKEFIAWLVKGRPSSGAPPPSGAP

SEQ ID NO: 41 - protein, 45 aa, synthetic construct
  REGION 1..45: note = Description of Artificial Sequence: Note = Synthetic Construct
HGEGTFTSDVSSYLEGQAAKEFIAWLVKGRPSSGAPPPSGAPPSS

SEQ ID NO: 42 - protein, 40 aa, synthetic construct
  REGION 1..40: note = Description of Artificial Sequence: Note = Synthetic Construct
  VARIANT 2: note = Xaa= aminohexanoic acid
HXAEGTFTSDVSSYLEGQAAKEFIAWLVKGRPSSGAPPPS

SEQ ID NO: 43 - protein, 43 aa, synthetic construct
  REGION 1..43: note = Description of Artificial Sequence: Note = Synthetic Construct
  VARIANT 2: note = Xaa= aminohexanoic acid
HXAEGTFTSDVSSYLEGQAAKEFIAWLVKGRPSSGAPPPSGAP

SEQ ID NO: 44 - protein, 46 aa, synthetic construct
  REGION 1..46: note = Description of Artificial Sequence: Note = Synthetic Construct
  VARIANT 2: note = Xaa= aminohexanoic acid
HXAEGTFTSDVSSYLEGQAAKEFIAWLVKGRPSSGAPPPSGAPPSS

SEQ ID NO: 45 - protein, 40 aa, synthetic construct
  REGION 1..40: note = Description of Artificial Sequence: Note = Synthetic Construct
  VARIANT 3: note = Xaa= aminohexanoic acid
HAXEGTFTSDVSSYLEGQAAKEFIAWLVKGRPSSGAPPPS

SEQ ID NO: 46 - protein, 43 aa, synthetic construct
  REGION 1..43: note = Description of Artificial Sequence: Note = Synthetic Construct
  VARIANT 3: note = Xaa= aminohexanoic acid
HAXEGTFTSDVSSYLEGQAAKEFIAWLVKGRPSSGAPPPSGAP

SEQ ID NO: 47 - protein, 46 aa, synthetic construct
  REGION 1..46: note = Description of Artificial Sequence: Note = Synthetic Construct
  VARIANT 3: note = Xaa= aminohexanoic acid
HAXEGTFTSDVSSYLEGQAAKEFIAWLVKGRPSSGAPPPSGAPPSS

SEQ ID NO: 48 - protein, 43 aa, synthetic construct
  REGION 1..43: note = Description of Artificial Sequence: Note = Synthetic Construct
  VARIANT 2: note = Xaa= aminohexanoic acid
YXAEGTFISDYSIAMDKIHQQDFVNWLLAQKGKKNDWKHNITQ

SEQ ID NO: 49 - protein, 36 aa, synthetic construct
  REGION 1..36: note = Description of Artificial Sequence: Note = Synthetic Construct
HGEGTFTSDLSKQMEEEAVRLFIEWLKNGGPSSGAP

SEQ ID NO: 50 - protein, 39 aa, synthetic construct; identical to SEQ ID NO: 39
  REGION 1..39: note = Description of Artificial Sequence: Note = Synthetic Construct

SEQ ID NO: 51 - protein, 36 aa, synthetic construct
  REGION 1..36: note = Description of Artificial Sequence: Note = Synthetic Construct
HGEGTFTSDVSSYLEGQAAKEFIAWLVKGRPSSGAP

SEQ ID NO: 52 - protein, 33 aa, synthetic construct
  REGION 1..33: note = Description of Artificial Sequence: Note = Synthetic Construct
HGEGTFTSDVSSYLEGQAAKEFIAWLVKGRPSS

SEQ ID NO: 53 - protein, 39 aa, synthetic construct
  REGION 1..39: note = amino acid sequence of Exendin-3
HSDGTFTSDLSKQMEEEAVRLFIEWLKNGGPSSGAPPPS

SEQ ID NO: 54 - protein, 31 aa, synthetic construct
  REGION 1..31: note = amino acid sequence of Exendin-4 variant
HGEGTFTSDLSKQMEEEAVRLFIEWLKNGGP

SEQ ID NO: 55 - protein, 39 aa, synthetic construct
  REGION 1..39: note = amino acid sequence of 14Leu25Phe Exendin-4 variant
HGEGTFTSDLSKQLEEEAVRLFIEFLKNGGPSSGAPPPS